European Patent Application EP 4 212 155 A1, published July 19, 2023. Title: Anti-senescence plant polyphenol drug downregulating senescence-related secretory phenotype and use thereof. Applicant: BY HEALTH CO LTD. Application EP 21923878.9, filed February 23, 2021. The sequence listing filed with the application follows.

SEQUENCE LISTING (28 sequences)

SEQ ID NO: 1 - DNA, 20 bp, synthetic construct
  misc_feature 1..20: note = IL6-F
  source 1..20: mol_type = other DNA
ttctgcgcagctttaaggag

SEQ ID NO: 2 - DNA, 20 bp, synthetic construct
  misc_feature 1..20: note = IL6-R
  source 1..20: mol_type = other DNA
aggtgcccatgctacatttg

SEQ ID NO: 3 - DNA, 21 bp, synthetic construct
  misc_feature 1..21: note = CXCL8-F
  source 1..21: mol_type = other DNA
atgacttccaagctggccgtg

SEQ ID NO: 4 - DNA, 20 bp, synthetic construct
  misc_feature 1..20: note = CXCL8-R
  source 1..20: mol_type = other DNA
tgtgttggcgcagtgtggtc

SEQ ID NO: 5 - DNA, 20 bp, synthetic construct
  misc_feature 1..20: note = SPINK1-F
  source 1..20: mol_type = other DNA
ccttggccctgttgagtcta

SEQ ID NO: 6 - DNA, 20 bp, synthetic construct
  misc_feature 1..20: note = SPINK1-R
  source 1..20: mol_type = other DNA
gcccagatttttgaatgagg

SEQ ID NO: 7 - DNA, 20 bp, synthetic construct
  misc_feature 1..20: note = WNT16B-F
  source 1..20: mol_type = other DNA
gctcctgtgctgtgaaaaca

SEQ ID NO: 8 - DNA, 20 bp, synthetic construct
  misc_feature 1..20: note = WNT16B-R
  source 1..20: mol_type = other DNA
tgcattctctgccttgtgtc

SEQ ID NO: 9 - DNA, 20 bp, synthetic construct
  misc_feature 1..20: note = GM-CSF-F
  source 1..20: mol_type = other DNA
atgtgaatgccatccaggag

SEQ ID NO: 10 - DNA, 20 bp, synthetic construct
  misc_feature 1..20: note = GM-CSF-R
  source 1..20: mol_type = other DNA
agggcagtgctgcttgtagt

SEQ ID NO: 11 - DNA, 20 bp, synthetic construct
  misc_feature 1..20: note = MMP3-F
  source 1..20: mol_type = other DNA
agggaacttgagcgtgaatc

SEQ ID NO: 12 - DNA, 20 bp, synthetic construct
  misc_feature 1..20: note = MMP3-R
  source 1..20: mol_type = other DNA
tcacttgtctgttgcacacg

SEQ ID NO: 13 - DNA, 20 bp, synthetic construct
  misc_feature 1..20: note = IL-1 alpha-F
  source 1..20: mol_type = other DNA
aatgacgccctcaatcaaag

SEQ ID NO: 14 - DNA, 20 bp, synthetic construct
  misc_feature 1..20: note = IL-1 alpha-R
  source 1..20: mol_type = other DNA
tgggtatctcaggcatctcc

SEQ ID NO: 15 - DNA, 18 bp, synthetic construct
  misc_feature 1..18: note = p16INK4a-F
  source 1..18: mol_type = other DNA
cttcctggacacgctggt

SEQ ID NO: 16 - DNA, 20 bp, synthetic construct
  misc_feature 1..20: note = p16INK4a-R
  source 1..20: mol_type = other DNA
atctatgcgggcatggttac

SEQ ID NO: 17 - DNA, 20 bp, synthetic construct
  misc_feature 1..20: note = IL-1 beta-F
  source 1..20: mol_type = other DNA
tgggtatctcaggcatctcc

SEQ ID NO: 18 - DNA, 20 bp, synthetic construct
  misc_feature 1..20: note = IL-1 beta-R
  source 1..20: mol_type = other DNA
ttctgcttgagaggtgctga

SEQ ID NO: 19 - DNA, 20 bp, synthetic construct
  misc_feature 1..20: note = AREG-F
  source 1..20: mol_type = other DNA
agctgcctttatgtctgctg

SEQ ID NO: 20 - DNA, 20 bp, synthetic construct
  misc_feature 1..20: note = AREG-R
  source 1..20: mol_type = other DNA
tttcgttcctcagcttctcc

SEQ ID NO: 21 - DNA, 20 bp, synthetic construct
  misc_feature 1..20: note = CXCL1-F
  source 1..20: mol_type = other DNA
caccccaagaacatccaaag

SEQ ID NO: 22 - DNA, 20 bp, synthetic construct
  misc_feature 1..20: note = CXCL1-R
  source 1..20: mol_type = other DNA
taactatgggggatgcagga

SEQ ID NO: 23 - DNA, 20 bp, synthetic construct
  misc_feature 1..20: note = CXCL3-F
  source 1..20: mol_type = other DNA
ggagcaccaactgacaggag

SEQ ID NO: 24 - DNA, 20 bp, synthetic construct
  misc_feature 1..20: note = CXCL3-R
  source 1..20: mol_type = other DNA
cctttccagctgtccctaga

SEQ ID NO: 25 - DNA, 20 bp, synthetic construct
  misc_feature 1..20: note = p21CIP1-F
  source 1..20: mol_type = other DNA
atgaaattcaccccctttcc

SEQ ID NO: 26 - DNA, 20 bp, synthetic construct
  misc_feature 1..20: note = p21CIP1-R
  source 1..20: mol_type = other DNA
ccctaggctgtgctcacttc

SEQ ID NO: 27 - DNA, 20 bp, synthetic construct
  misc_feature 1..20: note = BMP6-F
  source 1..20: mol_type = other DNA
aagaaggctggctggaattt

SEQ ID NO: 28 - DNA, 20 bp, synthetic construct
  misc_feature 1..20: note = BMP6-R
  source 1..20: mol_type = other DNA
gaagggctgcttgtcgtaag